European Patent Application EP 4 154 913 A1, published March 29, 2023. Title: Conjugates of Glucagon and AMPK activators. Applicant: University of Copenhagen. The sequence listing filed with the application follows.

SEQUENCE LISTING (2 sequences)

SEQ ID NO: 1 - protein, 40 aa, Homo sapiens
  Glucagon modified
  VARIANT 2: D-alanine, D-serine, alpha-aminoisobutyric acid, N-methyl-serine, glycine, or valine
  VARIANT 40: L-penicillamine or L-homocysteine
HSQGTFTSDYSKYLDSRRAQDFVQWLMNGGPSSGAPPPSC

SEQ ID NO: 2 - protein, 29 aa, Homo sapiens
  Glucagon unmodified
HSQGTFTSDYSKYLDSRRAQDFVQWLMNT